European Patent Specification EP 3 310 904 B1, published April 3, 2024. Title: Cellular Targeted Active Ingredient Delivery System. Applicant: Cellis Sp. Z o.o. The sequence listing filed with the application follows.

SEQUENCE LISTING (28 sequences)

SEQ ID NO: 1 - protein, 132 aa, Artificial Sequence
  Minimal consensus sequence of mammalian ferritin H chain
  MISC_FEATURE (5)..(5): Xaa at position 5 may be present or absent, if present it means any naturally occurring amino acid, preferably Ile
  MISC_FEATURE (6)..(6): Xaa at position 6 means any naturally occurring amino acid, preferably Asn
  MISC_FEATURE (14)..(14): Xaa at position 14 means any naturally occurring amino acid, preferably Tyr
  MISC_FEATURE (24)..(24): Xaa at position 24 means any naturally occurring amino acid, preferably Tyr or Cys, more preferably Tyr
  MISC_FEATURE (66)..(66): Xaa at position 66 means any naturally occurring amino acid, preferably Phe
  MISC_FEATURE (68)..(68): Xaa at position 68 means any naturally occurring amino acid, preferably Gln
  MISC_FEATURE (75)..(75): Xaa at position 75 means any naturally occurring amino acid, preferably Arg or Cys, more preferably Cys
  MISC_FEATURE (90)..(90): Xaa at position 90 means any naturally occurring amino acid, preferably His
  MISC_FEATURE (94)..(94): Xaa at position 94 means any naturally occurring amino acid, preferably Ser or Asn, more preferably Asn
  MISC_FEATURE (120)..(120): Xaa at position 120 may be present or absent, if present it means any naturally occurring amino acid, preferably His or Tyr, more preferably His
  MISC_FEATURE (123)..(123): Xaa at position 123 means any naturally occurring amino acid, preferably Asn or Ser, more preferably Asn
  MISC_FEATURE (128)..(128): Xaa at position 128 means any naturally occurring amino acid, preferably Ala or Ser, more preferably Ala
SEAAXXRQINLELXASYVYLSMSXYFDRDDVALKNFAKYFLHQSHEEREHAEKLMKLQNQRGGRIXLXDIKKPDXDDWESGLNAMECALXLEKXNQSLLELHKLATDKNDPHLCDFIETXYLXEQVKXIKEL

SEQ ID NO: 2 - protein, 183 aa, Artificial Sequence
  Consensus sequence of mammalian ferritin H chain
  MISC_FEATURE (6)..(6): Xaa at position 6 can be any naturally occurring amino acid, preferably Pro
  MISC_FEATURE (14)..(14): Xaa at position 14 can be any naturally occurring amino acid, preferably His
  MISC_FEATURE (16)..(16): Xaa at position 16 can be any naturally occurring amino acid, preferably Asp
  MISC_FEATURE (21)..(21): Xaa at position 21 may be present or absent, if present it means any naturally occurring amino acid, preferably Ile
  MISC_FEATURE (22)..(22): Xaa at position 22  means any naturally occurring amino acid, preferably Asn
  MISC_FEATURE (30)..(30): Xaa at position 30 can be any naturally occurring amino acid, preferably Tyr
  MISC_FEATURE (40)..(40): Xaa at position 40 can be any naturally occurring amino acid, preferably Tyr or Cys, more preferably Tyr
  MISC_FEATURE (82)..(82): Xaa at position 82 can be any naturally occurring amino acid, preferably Phe
  MISC_FEATURE (84)..(84): Xaa at position 84 can be any naturally occurring amino acid, preferably Gln
  MISC_FEATURE (91)..(91): Xaa at position 91 can be any naturally occurring amino acid, preferably Arg or Cys, more preferably Cys
  MISC_FEATURE (106)..(106): Xaa at position 106 can be any naturally occurring amino acid, preferably His
  MISC_FEATURE (110)..(110): Xaa at position 110 can be any naturally occurring amino acid, preferably Asn or Ser, more preferably Asn
  MISC_FEATURE (137)..(137): Xaa at position 137 can be any naturally occurring amino acid, preferably His or Tyr, more preferably His
  MISC_FEATURE (140)..(140): Xaa at position 140 can be any naturally occurring amino acid, preferably Asn or Ser, more preferably Asn
  MISC_FEATURE (145)..(145): Xaa at position 145 can be any naturally occurring amino acid, preferably Ala or Ser, more preferably Ala
  MISC_FEATURE (164)..(164): Xaa at position 164 can be any naturally occurring amino acid, preferably Ala or Ser, more preferably Ser
  MISC_FEATURE (166)..(166): Xaa at position 166 can be any naturally occurring amino acid, preferably Met or Leu, prerferably Leu
  MISC_FEATURE (178)..(178): Xaa at position 178 can be any naturally occurring amino acid, preferably Asp or His, more preferably Asp
  MISC_FEATURE (181)..(181): Xaa at position 181 is absent or any naturally occurring amino acid, preferably Asn
  MISC_FEATURE (182)..(182): Xaa at position 182 is absent or any naturally occurring amino acid, preferably Glu
  MISC_FEATURE (183)..(183): Xaa at position 183 is absent or any naturally occurring amino acid, preferably Ser
MTTASXSQVRQNYXQXSEAAXXRQINLELXASYVYLSMSXYFDRDDVALKNFAKYFLHQSHEEREHAEKLMKLQNQRGGRIXLXDIKKPDXDDWESGLNAMECALXLEKXVNQSLLELHKLATDKNDPHLCDFIETXYLXEQVKXIKELGDHVTNLRKMGAPEXGXAEYLFDKHTLGXSDXXX

SEQ ID NO: 3 - protein, 133 aa, Mus musculus
AEAAINRQINLELYASYVYLSMSCYFDRDDVALKNFAKYFLHQSHEEREHAEKLMKLQNQRGGRIFLQDIKKPDRDDWESGLNAMECALHLEKSVNQSLLELHKLATDKNDPHLCDFIETYYLSEQVKSIKEL

SEQ ID NO: 4 - protein, 180 aa, Mus musculus
MTTASPSQVRQNYHQDAEAAINRQINLELYASYVYLSMSCYFDRDDVALKNFAKYFLHQSHEEREHAEKLMKLQNQRGGRIFLQDIKKPDRDDWESGLNAMECALHLEKSVNQSLLELHKLATDKNDPHLCDFIETYYLSEQVKSIKELGDHVTNLRKMGAPEAGMAEYLFDKHTLGHGD

SEQ ID NO: 5 - protein, 132 aa, Homo sapiens
SEAANRQINLELYASYVYLSMSYYFDRDDVALKNFAKYFLHQSHEEREHAEKLMKLQNQRGGRIFLQDIKKPDCDDWESGLNAMECALHLEKNVNQSLLELHKLATDKNDPHLCDFIETHYLNEQVKAIKEL

SEQ ID NO: 6 - protein, 179 aa, Homo sapiens
MTTASTSQVRQNYHQDSEAANRQINLELYASYVYLSMSYYFDRDDVALKNFAKYFLHQSHEEREHAEKLMKLQNQRGGRIFLQDIKKPDCDDWESGLNAMECALHLEKNVNQSLLELHKLATDKNDPHLCDFIETHYLNEQVKAIKELGDHVTNLRKMGAPESGLAEYLFDKHTLGDSD

SEQ ID NO: 7 - protein, 182 aa, Artificial Sequence
  Consensus sequence of mammalian ferritin H chains 2nd version
  MISC_FEATURE (6)..(6): Xaa at position 6 can be any naturally occurring amino acid, preferably Pro
  MISC_FEATURE (14)..(14): Xaa at position 14 can be any naturally occurring amino acid, preferably His
  MISC_FEATURE (16)..(16): Xaa at position 16 can be any naturally occurring amino acid, preferably Asp
  MISC_FEATURE (21)..(21): Xaa at position 21 may be present or absent, if present it means any naturally occurring amino acid, preferably Ile
  MISC_FEATURE (29)..(29): Xaa at position 29 can be any naturally occurring amino acid, preferably Tyr
  MISC_FEATURE (81)..(81): Xaa at position 81 can be any naturally occurring amino acid, preferably Phe
  MISC_FEATURE (83)..(83): Xaa at position 83 can be any naturally occurring amino acid, preferably Gln
  MISC_FEATURE (105)..(105): Xaa at position 105 can be any naturally occurring amino acid, preferably His
  MISC_FEATURE (144)..(144): Xaa at position 144 can be any naturally occurring amino acid, preferably Ala or Ser, more preferably Ala
  MISC_FEATURE (180)..(180): Xaa at position 180 is absent or any naturally occuring amino acid, preferably Asn
  MISC_FEATURE (181)..(181): Xaa at position 181 is absent or any naturally occuring amino acid, preferably Glu
  MISC_FEATURE (182)..(182): Xaa at position 182 is absent or any naturally occuring amino acid, preferably Ser
MTTASXSQVRQNYXQXSEAAXRQINLELXASYVYLSMSYYFDRDDVALKNFAKYFLHQSHEEREHAEKLMKLQNQRGGRIXLXDIKKPDCDDWESGLNAMECALXLEKNVNQSLLELHKLATDKNDPHLCDFIETHYLNEQVKXIKELGDHVTNLRKMGAPESGLAEYLFDKHTLGDSDXXX

SEQ ID NO: 8 - protein, 150 aa, Artificial Sequence
  Minimal consensus sequence of mammalian ferritin L chain
  MISC_FEATURE (5)..(5): Xaa at position 5 can be any naturally occurring amino acid, preferably Asp or Glu, more preferably Asp
  MISC_FEATURE (12)..(12): Xaa at position 12 can be any nnaturally occurring amino acid, preferably Arg or Ser, more preferably Ser
  MISC_FEATURE (17)..(17): Xaa at position 17 can be any naturally occurring amino acid, preferably Ser or Arg, more preferably Ser
  MISC_FEATURE (19)..(19): Xaa at position 19 can be any naturally occurring amino acid, preferably Arg or Gln, more preferably Gln
  MISC_FEATURE (29)..(29): Xaa at position 29 can be any naturally occurring amino acid, preferably Phe
  MISC_FEATURE (30)..(30): Xaa at position 30 can be any naturally occurring amino acid, preferably Tyr or Phe, more preferably Tyr
  MISC_FEATURE (42)..(42): Xaa at position 42 can be any naturally occurring amino acid, preferably Ser or Gly, more preferably Ser
  MISC_FEATURE (56)..(56): Xaa at position 56 can be any naturally occurirng amino acid, preferably Ala or Tyr, more preferably Tyr
  MISC_FEATURE (61)..(61): Xaa at position 61 can be any naturally occurring amino acid, preferably Glu or Lys, more preferably Lys
  MISC_FEATURE (62)..(62): Xaa at position 62 can be any naturally occurring amino acid, preferably Met or Phe, more preferably Met
  MISC_FEATURE (65)..(65): Xaa at position 65 can be any naturally occurring amino acid, preferably Asp or Gln, more preferably Gln
  MISC_FEATURE (75)..(75): Xaa at position 75 can be any naturally occurring amino acid, preferably Ile or Val, more preferably Ile
  MISC_FEATURE (76)..(76): Xaa at position 76 can be any naturally occurring amino acid, preferably Lys or Gln, more preferably Lys
  MISC_FEATURE (79)..(79): Xaa at position 79 can be any naturally occurring amino acid, preferably Ala or Ser, more preferably Ala
  MISC_FEATURE (80)..(80): Xaa at position 80 can be any naturally occurring amino acid, preferably Glu or Gln, more preferably Gln
  MISC_FEATURE (87)..(87): Xaa at position 87 can be any naturally occurring amino acid, preferably Pro or Gln, more preferably Pro
  MISC_FEATURE (88)..(88): Xaa at position 88 can be any naturally occurring amino acid, preferably Glu or Asp, more preferably Asp
  MISC_FEATURE (91)..(91): Xaa at position 91 can be any naturally occurring amino acid, preferably Glu or Lys, more preferably Lys
  MISC_FEATURE (94)..(94): Xaa at position 94 can be any naturally occurring amino acid, preferably Met or Leu, more preferably Leu
  MISC_FEATURE (96)..(96): Xaa at position 96 can be any naturally occurring amino acid, preferably Met or Leu, more preferably Met
  MISC_FEATURE (99)..(99): Xaa at position 99 can be any naturally occurring amino acid, preferably Lys or Asn, preferably Lys
  MISC_FEATURE (115)..(115): Xaa at position 115 can be any naturally occurring amino acid, preferably Thr or Ala, more preferably Thr
  MISC_FEATURE (119)..(119): Xaa at position 119 can be any naturally occurring amino acid, preferably Leu
  MISC_FEATURE (125)..(125): Xaa at position 125 can be any naturally occurring amino acid, preferably Ser or Thr, more preferably Thr
  MISC_FEATURE (127)..(127): Xaa at position 127 can be any naturally occurring amino acid, preferably Tyr or Phe, more preferably Phe
  MISC_FEATURE (130)..(130): Xaa at position 130 can be any naturally occurring amino acid, preferably Lys or Glu, more preferably Glu
  MISC_FEATURE (140)..(140): Xaa at position 140 can be any naturally occurring amino acid, preferably Asp or Asn, more preferably Asp
  MISC_FEATURE (146)..(146): Xaa at position 146 can be any naturally occurring amino acid, preferably Arg or His, more preferably His
  MISC_FEATURE (148)..(148): Xaa at position 148 can be any naturally occurring amino acid, preferably Leu or Val, more preferably Leu
NYSTXVEAAVNXLVNLXLXASYTYLSLGXXFDRDDVALEGVXHFFRELAEEKREGXERLLXXQNXRGGRALFQDXXKPXXDEWGKTXXAMXAAXAXEKXLNQALLDLHALGSARXDPHXCDFLEXHXLDXEVKLIKKMGXHLTNLXRXAG

SEQ ID NO: 9 - protein, 183 aa, Artificial Sequence
  Consensus sequence of mammalian ferritin L chain
  MISC_FEATURE (12)..(12): Xaa at position 12 can be any naturally occurring amino acid, preferably Asp or Glu, more preferably Asp
  MISC_FEATURE (19)..(19): Xaa at position 19 can be any naturally occurring amino acid, preferably Ser or Arg, more preferably Ser
  MISC_FEATURE (24)..(24): Xaa at position 24 can be any naturally occurring amino acid, preferably Ser or Arg, more preferably Ser
  MISC_FEATURE (26)..(26): Xaa at position 26 can be any naturally occurring amino acid, preferably Arg or Gln, more preferably Gln
  MISC_FEATURE (36)..(36): Xaa at position 36 can be any naturally occurring amino acid, preferably Phe
  MISC_FEATURE (37)..(37): Xaa at position 37 can be any naturally occurring amino acid, preferably Tyr or Phe, more preferably Tyr
  MISC_FEATURE (49)..(49): Xaa at position 47 can be any naturally occurring amino acid, preferably Ser or Gly, more preferably Ser
  MISC_FEATURE (63)..(63): Xaa at position 63 can be any naturally occurring amino acid, preferably Ala or Tyr, more preferably Tyr
  MISC_FEATURE (68)..(68): Xaa at position 68 can be any naturally occurring amino acid, preferably Glu or Lys, more preferably Lys
  MISC_FEATURE (69)..(69): Xaa at position 69 can be any naturally occurring amino acid, preferably Met or Phe, more preferably Met
  MISC_FEATURE (72)..(72): Xaa at position 72 can be any naturally occurring amino acid, preferably Asp or Gln, more preferably Gln
  MISC_FEATURE (82)..(82): Xaa at position 82 can be any naturally occurring amino acid, preferably Ile or Val, more preferably Ile
  MISC_FEATURE (83)..(83): Xaa at position 83 can be any naturally occurring amino acid, preferably Lys or Gln, more preferably Lys
  MISC_FEATURE (86)..(86): Xaa at position 86 can be any naturally occurring amino acid, preferably Ala or Ser, more preferably Ala
  MISC_FEATURE (87)..(87): Xaa at position 87 can be any naturally occurring amino acid, preferably Glu or Gln, more preferably Gln
  MISC_FEATURE (94)..(94): Xaa at position 94 can be any naturally occurring amino acid, preferably Pro or Gln, more preferably Pro
  MISC_FEATURE (95)..(95): Xaa at position 95 can be any naturally occurring amino acid, preferably Glu or Asp, more preferably Asp
  MISC_FEATURE (98)..(98): Xaa at position 98 can be any naturally occurring amino acid, preferably Glu or Lys, more preferably Lys
  MISC_FEATURE (101)..(101): Xaa at position 101 can be any naturally occurring amino acid, preferably Met or Leu, more preferably Leu
  MISC_FEATURE (103)..(103): Xaa at position 103 can be any naturally occurring amino acid, preferably Met or Leu, more preferably Met
  MISC_FEATURE (106)..(106): Xaa at position 106 can be any naturally occurring amino acid, preferably Lys or Asn, preferably Lys
  misc_feature (122)..(122): Xaa can be any naturally occurring amino acid
  MISC_FEATURE (126)..(126): Xaa at position 126 can be any naturally occurring  amino acid, preferably Leu
  MISC_FEATURE (132)..(132): Xaa at position 132 can be any naturally occurring amino acid, preferably Ser or Thr, more preferably Thr
  MISC_FEATURE (134)..(134): Xaa at position 134 can be any naturally occurring amino acid, preferably Tyr or Phe, more preferably Phe
  MISC_FEATURE (137)..(137): Xaa at position 137 can be any naturally occurring amino acid, preferably Lys or Glu, more preferably Glu
  MISC_FEATURE (147)..(147): Xaa at position 147 can be any naturally occurring amino acid, preferably Asp or Asn, more preferably Asp
  MISC_FEATURE (153)..(153): Xaa at position 153 can be any naturally occurring amino acid, preferably Arg or His, more preferably His
  MISC_FEATURE (155)..(155): Xaa at position 155 can be any naturally occurring  amino acid, preferably Leu or Val, more preferably Leu
  MISC_FEATURE (161)..(161): Xaa at position 161 can be absent or any naturally occurring amino acid, preferably Ala
  MISC_FEATURE (163)..(163): Xaa at position 163 can be absent or any naturally occurring amino acid, preferably Thr
  MISC_FEATURE (166)..(166): Xaa at position 166 can be absent or any naturally occurring amino acid, preferably Pro
  MISC_FEATURE (168)..(168): Xaa at position 168 can be any naturally occurring amino acid, preferably Gly or Ala, more preferably Ala
MTSQIRQNYSTXVEAAVNXLVNLXLXASYTYLSLGXXFDRDDVALEGVXHFFRELAEEKREGXERLLXXQNXRGGRALFQDXXKPXXDEWGKTXXAMXAAXAXEKXLNQALLDLHALGSARXDPHXCDFLEXHXLDXEVKLIKKMGXHLTNLXRXAGPQPXQXGVXQXSLGEYLFERLTLKHD

SEQ ID NO: 10 - protein, 150 aa, Mus musculus
  MISC_FEATURE (12)..(12): Xaa at position 5 can be any naturally occuring amino acid, preferably Asp or Glu, more preferably Asp
NYSTEVEAAVNRLVNLHLRASYTYLSLGFFFDRDDVALEGVGHFFRELAEEKREGAERLLEFQNDRGGRALFQDVQKPSQDEWGKTQEAMEAALAMEKNLNQALLDLHALGSARADPHLCDFLESHYLDKEVKLIKKMGNHLTNLRRVAG

SEQ ID NO: 11 - skipped

SEQ ID NO: 12 - protein, 149 aa, Homo sapiens
NYSTDVEAAVNSLVNLYLQASYTYLSLGFYFDRDDVALEGVSHFFRELAEEKREGYERLLKMQNQRGGRALFQDIKKPAEDEWGKTPDAMKAAMALEKKLNQALLDLHALGSARTDPHLCDFLETHFLDEEVKLIKKMGDHLTNLHRLG

SEQ ID NO: 13 - protein, 175 aa, Homo sapiens
MSSQIRQNYSTDVEAAVNSLVNLYLQASYTYLSLGFYFDRDDVALEGVSHFFRELAEEKREGYERLLKMQNQRGGRALFQDIKKPAEDEWGKTPDAMKAAMALEKKLNQALLDLHALGSARTDPHLCDFLETHFLDEEVKLIKKMGDHLTNLHRLGGPEAGLGEYLFERLTLKHD

SEQ ID NO: 14 - protein, 183 aa, Artificial Sequence
  Consensus seqeuence of mammaliam ferritin L chain 2nd version
  MISC_FEATURE (36)..(36): Xaa at position 36 can be any naturally occuring amino acid, preferably Phe
  MISC_FEATURE (37)..(37): Xaa at position 37 can be any naturally occuring amino acid, preferably Tyr or Phe, more preferably Tyr
  MISC_FEATURE (94)..(94): Xaa at position 94 can be any naturally occurring  amino acid, preferably Pro or Gln, more preferably Pro
  MISC_FEATURE (126)..(126): Xaa at position 126 can be any naturally occurring  amino acid, preferably Leu
  MISC_FEATURE (137)..(137): Xaa at position 137 can be any naturally occurring  amino acid, preferably Lys or Glu, more preferably Glu
  MISC_FEATURE (147)..(147): Xaa at position 147 can be any naturally occurring  amino acid, preferably Asp or Asn, more preferably Asp
  misc_feature (161)..(161): Xaa can be any naturally occurring amino acid
  MISC_FEATURE (163)..(163): Xaa at position 163 can be absent or any naturally occurring amino acid, preferably Thr
  MISC_FEATURE (166)..(166): Xaa at position 166 can be absent or any naturally occurring amino acid, preferably Pro
  MISC_FEATURE (168)..(168): Xaa at position 168 can be any naturally occurring  amino acid, preferably Gly or Ala, more preferably Ala
MTSQIRQNYSTEVEAAVNRLVNLHLRASYTYLSLGXXFDRDDVALEGVGHFFRELAEEKREGAERLLKLQNQRGGRALFQDVQKPAQDEWGKTXEAMEAALALEKNLNQALLDLHALGSARTDPHXCDFLENHFLDXEVKLIKKMGXHLTNLRRLAGPQPXQXGVXQXSLGEYLFERLTLKHD

SEQ ID NO: 15 - protein, 117 aa, Artificial Sequence
  Minimal consensus sequence of mammalian haemoglobin alpha chain
  MISC_FEATURE (5)..(5): Xaa can be any naturally occurring amino acid, preferably Ala
  MISC_FEATURE (9)..(9): Xaa can be any naturally occurring amino acid, preferably Gly
  MISC_FEATURE (15)..(15): Xaa can be any naturally occurring amino acid, preferably Arg
  MISC_FEATURE (21)..(21): Xaa can be any naturally occurring amino acid, preferably Pro
  MISC_FEATURE (22)..(22): Xaa can be any naturally occurring amino acid, preferably Thr
  MISC_FEATURE (38)..(38): Xaa can be any naturally occurring amino acid, preferably Gln
  MISC_FEATURE (41)..(41): Xaa can be any naturally occurring amino acid, preferably Gly
  MISC_FEATURE (48)..(48): Xaa can be any naturally occurring amino acid, preferably Asp
  MISC_FEATURE (49)..(49): Xaa can be any naturally occurring amino acid, preferably Ala
  MISC_FEATURE (55)..(55): Xaa can be any naturally occurring amino acid, preferably Ala
  MISC_FEATURE (59)..(59): Xaa can be any naturally occurring amino acid, preferably Aap
  MISC_FEATURE (60)..(60): Xaa can be any naturally occurring amino acid, preferably Met
  MISC_FEATURE (68)..(68): Xaa can be any naturally occurring amino acid, preferably Ser
  MISC_FEATURE (76)..(76): Xaa can be any naturally occurring amino acid, preferably Arg
  MISC_FEATURE (79)..(79): Xaa can be any naturally occurring amino acid, preferably Pro
  MISC_FEATURE (90)..(90): Xaa can be any naturally occurring amino acid, preferably Leu
  MISC_FEATURE (91)..(91): Xaa can be any naturally occurring amino acid, preferably Val
  MISC_FEATURE (94)..(94): Xaa can be any naturally occurring amino acid, preferably Ala
  MISC_FEATURE (102)..(102): Xaa can be any naturally occurring amino acid, preferably Thr
  MISC_FEATURE (108)..(108): Xaa can be any naturally occurring amino acid, preferably Ser
  MISC_FEATURE (117)..(117): Xaa can be any naturally occurring amino acid, preferably Ser
VGAHXGEYXAEALEXMFLSFXXTKTYFPHFDLSHGSAXVKXHGKKVAXXLTNAVXHVDXXPNALSALXDLHAHKLXVDXVNFKLLSHCLXXTLXAHLPAEFXPAVHAXLDKFLASVX

SEQ ID NO: 16 - protein, 142 aa, Artificial Sequence
  Consensus sequence of mammalian alpha chain haemoglobins
  MISC_FEATURE (1)..(1): Xaa can be any naturally occurring amino acid, preferably Met
  MISC_FEATURE (2)..(2): Xaa can be any naturally occurring amino acid, preferably Val
  MISC_FEATURE (14)..(14): Xaa can be any naturally occurring amino acid, preferably Ala
  MISC_FEATURE (17)..(17): Xaa can be any naturally occurring amino acid, preferably Lys
  MISC_FEATURE (22)..(22): Xaa can be any naturally occurring amino acid, preferably Ala
  MISC_FEATURE (26)..(26): Xaa can be any naturally occurring amino acid, preferably Gly
  MISC_FEATURE (32)..(32): Xaa can be any naturally occurring amino acid, preferably Arg
  MISC_FEATURE (38)..(38): Xaa can be any naturally occurring amino acid, preferably Pro
  MISC_FEATURE (39)..(39): Xaa can be any naturally occurring amino acid, preferably Thr
  MISC_FEATURE (55)..(55): Xaa can be any naturally occurring amino acid, preferably Gln
  MISC_FEATURE (58)..(58): Xaa can be any naturally occurring amino acid, preferably Gly
  MISC_FEATURE (65)..(65): Xaa can be any naturally occurring amino acid, preferably Asp
  MISC_FEATURE (66)..(66): Xaa can be any naturally occurring amino acid, preferably Ala
  MISC_FEATURE (72)..(72): Xaa can be any naturally occurring amino acid, preferably Ala
  MISC_FEATURE (76)..(76): Xaa can be any naturally occurring amino acid, preferably Asp
  MISC_FEATURE (77)..(77): Xaa can be any naturally occurring amino acid, preferably Met
  MISC_FEATURE (85)..(85): Xaa can be any naturally occurring amino acid, preferably Ser
  MISC_FEATURE (93)..(93): Xaa can be any naturally occurring amino acid, preferably Arg
  MISC_FEATURE (96)..(96): Xaa can be any naturally occurring amino acid, preferably Pro
  MISC_FEATURE (107)..(107): Xaa can be any naturally occurring amino acid, preferably Leu
  MISC_FEATURE (108)..(108): Xaa can be any naturally occurring amino acid, preferably Val
  MISC_FEATURE (111)..(111): Xaa can be any naturally occurring amino acid, preferably Ala
  MISC_FEATURE (119)..(119): Xaa can be any naturally occurring amino acid, preferably Thr
  MISC_FEATURE (125)..(125): Xaa can be any naturally occurring amino acid, preferably Ser
  MISC_FEATURE (134)..(134): Xaa can be any naturally occurring amino acid, preferably Ser
  MISC_FEATURE (142)..(142): Xaa can be any naturally occurring amino acid, preferably Arg
XXLSPADKTNVKAXWGXVGAHXGEYXAEALEXMFLSFXXTKTYFPHFDLSHGSAXVKXHGKKVAXXLTNAVXHVDXXPNALSALXDLHAHKLXVDXVNFKLLSHCLXXTLXAHLPAEFXPAVHAXLDKFLASVXTVLTSKYX

SEQ ID NO: 17 - protein, 117 aa, Homo sapiens
VGAHAGEYGAEALERMFLSFPTTKTYFPHFDLSHGSAQVKGHGKKVADALTNAVAHVDDMPNALSALSDLHAHKLRVDPVNFKLLSHCLLVTLAAHLPAEFTPAVHASLDKFLASVS

SEQ ID NO: 18 - protein, 142 aa, Homo sapiens
MVLSPADKTNVKAAWGKVGAHAGEYGAEALERMFLSFPTTKTYFPHFDLSHGSAQVKGHGKKVADALTNAVAHVDDMPNALSALSDLHAHKLRVDPVNFKLLSHCLLVTLAAHLPAEFTPAVHASLDKFLASVSTVLTSKYR

SEQ ID NO: 19 - protein, 124 aa, Artificial Sequence
  Minimal consensus sequence of mammalian haemoglobin beta chain
  MISC_FEATURE (4)..(4): Xaa can be any naturally occurring amino acid, preferably Asn
  MISC_FEATURE (9)..(9): Xaa can be any naturally occurring amino acid, preferably Gly
  MISC_FEATURE (10)..(10): Xaa can be any naturally occurring amino acid, preferably Gly
  MISC_FEATURE (12)..(12): Xaa can be absent or any naturally occurring amino acid, preferably Ala
  MISC_FEATURE (13)..(13): Xaa can be absent or any naturally occurring amino acid, preferably Leu
  MISC_FEATURE (14)..(14): Xaa can be absent or any naturally occurring amino acid, preferably Gly
  MISC_FEATURE (15)..(15): Xaa can be absent or any naturally occurring amino acid, preferably Arg
  MISC_FEATURE (27)..(27): Xaa can be absent or any naturally occurring amino acid, preferably Leu
  MISC_FEATURE (35)..(35): Xaa can be absent or any naturally occurring amino acid, preferably Thr
  MISC_FEATURE (36)..(36): Xaa can be absent or any naturally occurring amino acid, preferably Pro
  MISC_FEATURE (49)..(49): Xaa can be absent or any naturally occurring amino acid, preferably Gly
  MISC_FEATURE (52)..(52): Xaa can be absent or any naturally occurring amino acid, preferably Val
  MISC_FEATURE (66)..(66): Xaa can be absent or any naturally occurring amino acid, preferably Leu
  MISC_FEATURE (68)..(68): Xaa can be absent or any naturally occurring amino acid, preferably Gly
  MISC_FEATURE (69)..(69): Xaa can be absent or any naturally occurring amino acid, preferably Thr
  MISC_FEATURE (86)..(86): Xaa can be absent or any naturally occurring amino acid, preferably Glu
  misc_feature (121)..(121): Xaa can be any naturally occurring amino acid
  MISC_FEATURE (122)..(122): Xaa can be absent or any naturally occurring amino acid, preferably Val
GKVXVDEVXXEXXXXLLVVYPWTQRFXESFGDLSXXDAVMGNPKVKAHXKKXLGAFSDGLAHLDNXKXXFATLSELHCDKLHVDPXNFRLLGNVLVCVLAHHFGKEFTPPVQAAYQKVVAXXAN

SEQ ID NO: 20 - protein, 147 aa, Artificial Sequence
  Consensus sequence of mammalian haemoglobin beta chain
  MISC_FEATURE (10)..(10): Xaa can be any naturally occurring amino acid, preferably Ser
  MISC_FEATURE (11)..(11): Xaa can be any naturally occurring amino acid, preferably Ala
  MISC_FEATURE (15)..(15): Xaa can be any naturally occurring amino acid, preferably Leu
  MISC_FEATURE (20)..(20): Xaa can be any naturally occurring amino acid, preferably Asn
  MISC_FEATURE (25)..(25): Xaa can be any naturally occurring amino acid, preferably Gly
  MISC_FEATURE (26)..(26): Xaa can be any naturally occurring amino acid, preferably Gly
  MISC_FEATURE (28)..(28): Xaa can be any naturally occurring amino acid, preferably Ala
  MISC_FEATURE (29)..(29): Xaa can be any naturally occurring amino acid, preferably Leu
  MISC_FEATURE (30)..(30): Xaa can be any naturally occurring amino acid, preferably Gly
  MISC_FEATURE (31)..(31): Xaa can be any naturally occurring amino acid, preferably Arg
  MISC_FEATURE (43)..(43): Xaa can be absent or any naturally occurring amino acid, preferably Leu
  MISC_FEATURE (51)..(51): Xaa can be any naturally occurring amino acid, preferably Thr
  MISC_FEATURE (52)..(52): Xaa can be any naturally occurring amino acid, preferably Pro
  MISC_FEATURE (65)..(65): Xaa can be any naturally occurring amino acid, preferably Gly
  MISC_FEATURE (68)..(68): Xaa can be any naturally occurring amino acid, preferably Val
  MISC_FEATURE (82)..(82): Xaa can be any naturally occurring amino acid, preferably Leu
  MISC_FEATURE (84)..(84): Xaa can be any naturally occurring amino acid, preferably Gly
  MISC_FEATURE (85)..(85): Xaa can be any naturally occurring amino acid, preferably Thr
  MISC_FEATURE (102)..(102): Xaa can be any naturally occurring amino acid, preferably Glu
  MISC_FEATURE (137)..(137): Xaa can be any naturally occurring amino acid, preferably Gly
  MISC_FEATURE (138)..(138): Xaa can be any naturally occurring amino acid, preferably Val
  MISC_FEATURE (147)..(147): Xaa can be any naturally occurring amino acid, preferably His
MVHLTPEEKXXVTAXWGKVXVDEVXXEXXXXLLVVYPWTQRFXESFGDLSXXDAVMGNPKVKAHXKKXLGAFSDGLAHLDNXKXXFATLSELHCDKLHVDPXNFRLLGNVLVCVLAHHFGKEFTPPVQAAYQKVVAXXANALAHKYX

SEQ ID NO: 21 - protein, 124 aa, Homo sapiens
GKVNVDEVGGEALGRLLVVYPWTQRFLESFGDLSTPDAVMGNPKVKAHGKKVLGAFSDGLAHLDNLKGTFATLSELHCDKLHVDPENFRLLGNVLVCVLAHHFGKEFTPPVQAAYQKVVAGVAN

SEQ ID NO: 22 - protein, 147 aa, Homo sapiens [sequence omitted]

SEQ ID NO: 23 - protein, 80 aa, Artificial Sequence
  N-terminal region of a consensus sequence of mammalian transferrins
  MISC_FEATURE (2)..(2): Xaa can be any naturally occurring amino acid, preferably Arg
  MISC_FEATURE (9)..(9): Xaa can be any naturally occurring amino acid, preferably Leu
  MISC_FEATURE (10)..(10): Xaa can be any naturally occurring amino acid, preferably Val
  MISC_FEATURE (15)..(15): Xaa can be any naturally occurring amino acid, preferably Gly
  MISC_FEATURE (24)..(24): Xaa can be any naturally occurring amino acid, preferably Thr
  MISC_FEATURE (25)..(25): Xaa can be any naturally occurring amino acid, preferably Val
  MISC_FEATURE (31)..(31): Xaa can be any naturally occurring amino acid, preferably Ser
  MISC_FEATURE (32)..(32): Xaa can be any naturally occurring amino acid, preferably Glu
  MISC_FEATURE (42)..(42): Xaa can be any naturally occurring amino acid, preferably Arg
  MISC_FEATURE (47)..(47): Xaa can be any naturally occurring amino acid, preferably Ser
  misc_feature (59)..(59): Xaa can be any naturally occurring amino acid
  MISC_FEATURE (64)..(64): Xaa can be any naturally occurring amino acid, preferably Tyr
  MISC_FEATURE (65)..(65): Xaa can be any naturally occurring amino acid, preferably Leu
  MISC_FEATURE (71)..(71): Xaa can be any naturally occurring amino acid, preferably Ile
  MISC_FEATURE (73)..(73): Xaa can be any naturally occurring amino acid, preferably Ala
  MISC_FEATURE (77)..(77): Xaa can be any naturally occurring amino acid, preferably Asp
  MISC_FEATURE (78)..(78): Xaa can be any naturally occurring amino acid, preferably Ala
MXLAVGALXXCAVLXLCLAVPDKXXRWCAVXXHEATKCQSFXDHMKXVIPSDGPSVACXKKASXXDCIRAXAXNEAXXVT

SEQ ID NO: 24 - protein, 114 aa, Artificial Sequence
  C-terminal region of a consensus sequence of mammalian transferrins
  MISC_FEATURE (3)..(3): Xaa can be any naturally occurring amino acid, preferably Thr
  MISC_FEATURE (16)..(16): Xaa can be any naturally occurring amino acid, preferably Asp
  MISC_FEATURE (18)..(18): Xaa can be any naturally occurring amino acid, preferably Met
  MISC_FEATURE (19)..(19): Xaa can be any naturally occurring amino acid, preferably Ser
  MISC_FEATURE (23)..(23): Xaa can be any naturally occurring amino acid, preferably Gly
  MISC_FEATURE (25)..(25): Xaa can be any naturally occurring amino acid, preferably Val
  MISC_FEATURE (28)..(28): Xaa can be any naturally occurring amino acid, preferably Ala
  MISC_FEATURE (30)..(30): Xaa can be any naturally occurring amino acid, preferably Lys
  MISC_FEATURE (61)..(61): Xaa can be any naturally occurring amino acid, preferably Val
  MISC_FEATURE (62)..(62): Xaa can be any naturally occurring amino acid, preferably Lys
  MISC_FEATURE (75)..(75): Xaa can be any naturally occurring amino acid, preferably Gly
  MISC_FEATURE (78)..(78): Xaa can be any naturally occurring amino acid, preferably Ser
  MISC_FEATURE (96)..(96): Xaa can be any naturally occurring amino acid, preferably Leu
  MISC_FEATURE (97)..(97): Xaa can be any naturally occurring amino acid, preferably Tyr
  MISC_FEATURE (105)..(105): Xaa can be any naturally occurring amino acid, preferably Phe
  MISC_FEATURE (107)..(107): Xaa can be any naturally occurring amino acid, preferably Glu
  MISC_FEATURE (110)..(110): Xaa can be any naturally occurring amino acid, preferably Ser
ETXEDCIAKIMNGEAXAXXLDGXFXYIXGXCGLVPVLAENYNKSDNCEDTPEAGYFAVAVXXKSASDLTWDNLKXKKXCHTAVGRTAGWNIPMGLXXNKINHCRXDXFFXEGCA

SEQ ID NO: 25 - protein, 698 aa, Artificial Sequence
  Consensus sequence of mammalian transferrins
  MISC_FEATURE (2)..(2): Xaa can be any naturally occurring amino acid, preferably Arg
  misc_feature (9)..(9): Xaa can be any naturally occurring amino acid
  MISC_FEATURE (10)..(10): Xaa can be any naturally occurring amino acid, preferably Val
  MISC_FEATURE (15)..(15): Xaa can be any naturally occurring amino acid, preferably Gly
  MISC_FEATURE (24)..(24): Xaa can be any naturally occurring amino acid, preferably Thr
  MISC_FEATURE (25)..(25): Xaa can be any naturally occurring amino acid, preferably Val
  MISC_FEATURE (31)..(31): Xaa can be any naturally occurring amino acid, preferably Ser
  MISC_FEATURE (32)..(32): Xaa can be any naturally occurring amino acid, preferably Glu
  MISC_FEATURE (42)..(42): Xaa can be any naturally occurring amino acid, preferably Arg
  MISC_FEATURE (47)..(47): Xaa can be any naturally occurring amino acid, preferably Ser
  MISC_FEATURE (59)..(59): Xaa can be any naturally occurring amino acid, preferably Val
  MISC_FEATURE (64)..(64): Xaa can be any naturally occurring amino acid, preferably Tyr
  MISC_FEATURE (65)..(65): Xaa can be any naturally occurring amino acid, preferably Leu
  misc_feature (71)..(71): Xaa can be any naturally occurring amino acid
  MISC_FEATURE (73)..(73): Xaa can be any naturally occurring amino acid, preferably Ile
  MISC_FEATURE (77)..(77): Xaa can be any naturally occurring amino acid, preferably Asp
  MISC_FEATURE (78)..(78): Xaa can be any naturally occurring amino acid, preferably Ala
  MISC_FEATURE (84)..(84): Xaa can be any naturally occurring amino acid, preferably Gly
  MISC_FEATURE (87)..(87): Xaa can be any naturally occurring amino acid, preferably Tyr
  MISC_FEATURE (88)..(88): Xaa can be any naturally occurring amino acid, preferably Asp
  MISC_FEATURE (94)..(94): Xaa can be any naturally occurring amino acid, preferably Asn
  MISC_FEATURE (98)..(98): Xaa can be any naturally occurring amino acid, preferably Pro
  MISC_FEATURE (104)..(104): Xaa can be any naturally occurring amino acid, preferably Tyr
  MISC_FEATURE (107)..(107): Xaa can be any naturally occurring amino acid, preferably Lys
  MISC_FEATURE (108)..(108): Xaa can be any naturally occurring amino acid, preferably Glu
  MISC_FEATURE (115)..(115): Xaa can be any naturally occurring amino acid, preferably Tyr
  MISC_FEATURE (116)..(116): Xaa can be any naturally occurring amino acid, preferably Ala
  MISC_FEATURE (121)..(121): Xaa can be any naturally occurring amino acid, preferably Lys
  MISC_FEATURE (124)..(124): Xaa can be any naturally occurring amino acid, preferably Ser
  MISC_FEATURE (129)..(129): Xaa can be any naturally occurring amino acid, preferably Asn
  MISC_FEATURE (146)..(146): Xaa can be any naturally occurring amino acid, preferably Gly
  MISC_FEATURE (152)..(152): Xaa can be any naturally occurring amino acid, preferably Gly
  MISC_FEATURE (153)..(153): Xaa can be any naturally occurring amino acid, preferably Leu
  MISC_FEATURE (161)..(161): Xaa can be any naturally occurring amino acid, preferably Pro
  MISC_FEATURE (179)..(179): Xaa can be any naturally occurring amino acid, preferably Pro
  MISC_FEATURE (188)..(188): Xaa can be any naturally occurring amino acid, preferably Gln
  MISC_FEATURE (204)..(204): Xaa can be any naturally occurring amino acid, preferably Tyr
  MISC_FEATURE (224)..(224): Xaa can be any naturally occurring amino acid, preferably Val
  MISC_FEATURE (238)..(238): Xaa can be any naturally occurring amino acid, preferably Asp
  MISC_FEATURE (245)..(245): Xaa can be any naturally occurring amino acid, preferably Leu
  MISC_FEATURE (255)..(255): Xaa can be any naturally occurring amino acid, preferably Asp
  MISC_FEATURE (268)..(268): Xaa can be any naturally occurring amino acid, preferably His
  MISC_FEATURE (275)..(275): Xaa can be any naturally occurring amino acid, preferably Met
  MISC_FEATURE (276)..(276): Xaa can be any naturally occurring amino acid, preferably Gly
  MISC_FEATURE (286)..(286): Xaa can be any naturally occurring amino acid, preferably Leu
  MISC_FEATURE (293)..(293): Xaa can be any naturally occurring amino acid, preferably Phe
  MISC_FEATURE (309)..(309): Xaa can be any naturally occurring amino acid, preferably Gly
  MISC_FEATURE (310)..(310): Xaa can be any naturally occurring amino acid, preferably Lys
  MISC_FEATURE (326)..(326): Xaa can be any naturally occurring amino acid, preferably Pro
  MISC_FEATURE (327)..(327): Xaa can be any naturally occurring amino acid, preferably Arg
  MISC_FEATURE (357)..(357): Xaa can be any naturally occurring amino acid, preferably Glu
  MISC_FEATURE (381)..(381): Xaa can be any naturally occurring amino acid, preferably Ser
  MISC_FEATURE (393)..(393): Xaa can be any naturally occurring amino acid, preferably Thr
  MISC_FEATURE (406)..(406): Xaa can be any naturally occurring amino acid, preferably Asp
  MISC_FEATURE (408)..(408): Xaa can be any naturally occurring amino acid, preferably Met
  MISC_FEATURE (409)..(409): Xaa can be any naturally occurring amino acid, preferably Ser
  MISC_FEATURE (413)..(413): Xaa can be any naturally occurring amino acid, preferably Gly
  MISC_FEATURE (415)..(415): Xaa can be any naturally occurring amino acid, preferably Val
  MISC_FEATURE (418)..(418): Xaa can be any naturally occurring amino acid, preferably Ala
  MISC_FEATURE (420)..(420): Xaa can be any naturally occurring amino acid, preferably Lys
  MISC_FEATURE (451)..(451): Xaa can be any naturally occurring amino acid, preferably Val
  MISC_FEATURE (452)..(452): Xaa can be any naturally occurring amino acid, preferably Lys
  MISC_FEATURE (465)..(465): Xaa can be any naturally occurring amino acid, preferably Gly
  MISC_FEATURE (468)..(468): Xaa can be any naturally occurring amino acid, preferably Ser
  MISC_FEATURE (486)..(486): Xaa can be any naturally occurring amino acid, preferably Leu
  MISC_FEATURE (487)..(487): Xaa can be any naturally occurring amino acid, preferably Tyr
  MISC_FEATURE (495)..(495): Xaa can be any naturally occurring amino acid, preferably Phe
  MISC_FEATURE (497)..(497): Xaa can be any naturally occurring amino acid, preferably Glu
  MISC_FEATURE (500)..(500): Xaa can be any naturally occurring amino acid, preferably Ser
  MISC_FEATURE (505)..(505): Xaa can be any naturally occurring amino acid, preferably Pro
  MISC_FEATURE (509)..(509): Xaa can be any naturally occurring amino acid, preferably Lys
  MISC_FEATURE (529)..(529): Xaa can be any naturally occurring amino acid, preferably Asn
  MISC_FEATURE (536)..(536): Xaa can be any naturally occurring amino acid, preferably Tyr
  MISC_FEATURE (558)..(558): Xaa can be any naturally occurring amino acid, preferably Pro
  misc_feature (559)..(559): Xaa can be any naturally occurring amino acid
  MISC_FEATURE (563)..(563): Xaa can be any naturally occurring amino acid, preferably Gly
  MISC_FEATURE (586)..(586): Xaa can be any naturally occurring amino acid, preferably Thr
  MISC_FEATURE (592)..(592): Xaa can be any naturally occurring amino acid, preferably Glu
  MISC_FEATURE (603)..(603): Xaa can be any naturally occurring amino acid, preferably Asn
  MISC_FEATURE (607)..(607): Xaa can be any naturally occurring amino acid, preferably Val
  MISC_FEATURE (622)..(622): Xaa can be any naturally occurring amino acid, preferably Gln
  MISC_FEATURE (635)..(635): Xaa can be any naturally occurring amino acid, preferably Ser
  MISC_FEATURE (648)..(648): Xaa can be any naturally occurring amino acid, preferably Leu
  MISC_FEATURE (652)..(652): Xaa can be any naturally occurring amino acid, preferably Asp
  MISC_FEATURE (678)..(678): Xaa can be any naturally occurring amino acid, preferably Val
  MISC_FEATURE (692)..(692): Xaa can be any naturally occurring amino acid, preferably Ala
  MISC_FEATURE (696)..(696): Xaa can be any naturally occurring amino acid, preferably Arg
  MISC_FEATURE (698)..(698): Xaa can be any naturally occurring amino acid, preferably Pro
MXLAVGALXXCAVLXLCLAVPDKXXRWCAVXXHEATKCQSFXDHMKXVIPSDGPSVACXKKASXXDCIRAXAXNEAXXVTLDAXLVXXAYLAPXNLKXVVAEFXGSXXDPQTFYXXVAVVXKDXGFQMXQLRGKKSCHTGLGRSAXWNIPIXXLYCDLPEXRKPLEKAVANFFSGSCAXCADGTDFPXLCQLCPGCGCSTLNQXFGYSGAFKCLKDGAGDVAFXKHSTIFENLANKAXRDQYELXCLDNTRKPVXEYKDCHLAQVPSXTVVARSXXGKEDLIWELXNQAQEHXGKDKSKEFQLFSSPHXXDLLFKDSAHGFLKVPXXMDAKMYLGYEYVTAIRNLREGTCPEAPTDXCKPVKWCALSHHERLKCDEWSVNXVGKIECVSAETXEDCIAKIMNGEAXAXXLDGXFXYIXGXCGLVPVLAENYNKSDNCEDTPEAGYFAVAVXXKSASDLTWDNLKXKKXCHTAVGRTAGWNIPMGLXXNKINHCRXDXFFXEGCAXGSKXDSSLCKLCMGSGLNLCEPNXKEGYYGXTGAFRCLVEKGDVAFVKHQTVXXNTGXKNPDPWAKNLNEKDYELLCLDGXRKPVEXYANCHLARAPXHAVXTRKDKEACVHKILRXQQHLFGSNVTDCXGNFCLFRSETKDXLFRXDTVCLAKLHDRNTYEKYLGEEYVKAXGNLRKCSTSSLLEXCTFXRX

SEQ ID NO: 26 - protein, 80 aa, Homo sapiens
MRLAVGALLVCAVLGLCLAVPDKTVRWCAVSEHEATKCQSFRDHMKSVIPSDGPSVACVKKASYLDCIRAIAANEADAVT

SEQ ID NO: 27 - protein, 114 aa, Homo sapiens
ETTEDCIAKIMNGEADAMSLDGGFVYIAGKCGLVPVLAENYNKSDNCEDTPEAGYFAVAVVKKSASDLTWDNLKGKKSCHTAVGRTAGWNIPMGLLYNKINHCRFDEFFSEGCA

SEQ ID NO: 28 - protein, 698 aa, Homo sapiens
MRLAVGALLVCAVLGLCLAVPDKTVRWCAVSEHEATKCQSFRDHMKSVIPSDGPSVACVKKASYLDCIRAIAANEADAVTLDAGLVYDAYLAPNNLKPVVAEFYGSKEDPQTFYYAVAVVKKDSGFQMNQLRGKKSCHTGLGRSAGWNIPIGLLYCDLPEPRKPLEKAVANFFSGSCAPCADGTDFPQLCQLCPGCGCSTLNQYFGYSGAFKCLKDGAGDVAFVKHSTIFENLANKADRDQYELLCLDNTRKPVDEYKDCHLAQVPSHTVVARSMGGKEDLIWELLNQAQEHFGKDKSKEFQLFSSPHGKDLLFKDSAHGFLKVPPRMDAKMYLGYEYVTAIRNLREGTCPEAPTDECKPVKWCALSHHERLKCDEWSVNSVGKIECVSAETTEDCIAKIMNGEADAMSLDGGFVYIAGKCGLVPVLAENYNKSDNCEDTPEAGYFAVAVVKKSASDLTWDNLKGKKSCHTAVGRTAGWNIPMGLLYNKINHCRFDEFFSEGCAPGSKKDSSLCKLCMGSGLNLCEPNNKEGYYGYTGAFRCLVEKGDVAFVKHQTVPQNTGGKNPDPWAKNLNEKDYELLCLDGTRKPVEEYANCHLARAPNHAVVTRKDKEACVHKILRQQQHLFGSNVTDCSGNFCLFRSETKDLLFRDDTVCLAKLHDRNTYEKYLGEEYVKAVGNLRKCSTSSLLEACTFRRP